European Patent Application EP 4 130 279 A1, published February 8, 2023. Title: Z DOMAIN-CALSEQUESTRIN FUSION PROTEIN WITH IMPROVED REACTIVITY ,STABILITY AND ANTIBODY RECOVERY AND METHOD OF ISOLATING AND PURIFYING ANTIBODY USING THE SAME. Applicant: Korea Institute of Ceramic Engineering and Technology. The sequence listing filed with the application follows.

SEQUENCE LISTING (14 sequences)

SEQ ID NO: 1 - protein, 116 aa, Artificial Sequence
  ZZ
VDNKFNKEQQNAFYEILHLPNLNEEQRNAFIQSLKDDPSQSANLLAEAKKLNDAQAPKVDNKFNKEQQNAFYEILHLPNLNEEQRNAFIQSLKDDPSQSANLLAEAKKLNDAQAPK

SEQ ID NO: 2 - protein, 132 aa, Artificial Sequence
  Z6G
VDNKFNKEQQNAFYEILHLPNLNEEQRNAFIQSLKDDPSQGGGGGGSANLLAEAKKLNDAQAPKVDVDNKFNKEQQNAFYEILHLPNLNEEQRNAFIQSLKDDPSQGGGGGGSANLLAEAKKLNDAQAPKVD

SEQ ID NO: 3 - protein, 120 aa, Artificial Sequence
  ZL4G
VDNKFNKEQQNAFYEILHLPNLNEEQRNAFIQSLKDGGGGSANLLAEAKKLNDAQAPKVDVDNKFNKEQQNAFYEILHLPNLNEEQRNAFIQSLKDGGGGSANLLAEAKKLNDAQAPKVD

SEQ ID NO: 4 - protein, 364 aa, Artificial Sequence
  CSQ2(delta)
EEGLNFPTYDGKDRVVSLSEKNFKQVLKKYDLLCLYYHEPVSSDKVTPKQFQLKEIVLELVAQVLEHKAIGFVMVDAKKEAKLAKKLGFDEEGSLYILKGDRTIEFDGEFAADVLVEFLLDLIEDPVEIISSKLEVQAFERIEDYIKLIGFFKSEDSEYYKAFEEAAEHFQPYIKFFATFDKGVAKKLSLKMNEVDFYEPFMDEPIAIPNKPYTEEELVEFVKEHQRPTLRRLRPEEMFETWEDDLNGIHIVAFAEKSDPDGYEFLEILKQVARDNTDNPDLSILWIDPDDFPLLVAYWEKTFKIDLFRPQIGVVNVTDADSVWMEIPDDDDLPTAEELEDWIEDVLSGKINTEDDDEDDDDDD

SEQ ID NO: 5 - protein, 362 aa, Artificial Sequence
  CSQ1(Full)
QEGLDFPEYDGVDRVINVNAKNYKNVFKKYEVLALLYHEPPEDDKASQRQFEMEELILELAAQVLEDKGVGFGLVDSEKDAAVAKKLGLTEVDSMYVFKGDEVIEYDGEFSADTIVEFLLDVLEDPVELIEGERELQAFENIEDEIKLIGYFKSKDSEHYKAFEDAAEEFHPYIPFFATFDSKVAKKLTLKLNEIDFYEAFMEEPVTIPDKPNSEEEIVNFVEEHRRSTLRKLKPESMYETWEDDMDGIHIVAFAEEADPDGFEFLETLKAVAQDNTENPDLSIIWIDPDDFPLLVPYWEKTFDIDLSAPQIGVVNVTDADSVWMEMDDEEDLPSAEELEDWLEDVLEGEINTEDDDDDDDD

SEQ ID NO: 6 - protein, 380 aa, Artificial Sequence
  CSQ2(Full)
EEGLNFPTYDGKDRVVSLSEKNFKQVLKKYDLLCLYYHEPVSSDKVTPKQFQLKEIVLELVAQVLEHKAIGFVMVDAKKEAKLAKKLGFDEEGSLYILKGDRTIEFDGEFAADVLVEFLLDLIEDPVEIISSKLEVQAFERIEDYIKLIGFFKSEDSEYYKAFEEAAEHFQPYIKFFATFDKGVAKKLSLKMNEVDFYEPFMDEPIAIPNKPYTEEELVEFVKEHQRPTLRRLRPEEMFETWEDDLNGIHIVAFAEKSDPDGYEFLEILKQVARDNTDNPDLSILWIDPDDFPLLVAYWEKTFKIDLFRPQIGVVNVTDADSVWMEIPDDDDLPTAEELEDWIEDVLSGKINTEDDDEDDDDDDNSDEEDNDDSDDDDDE

SEQ ID NO: 7 - protein, 10 aa, Artificial Sequence
  G4S
GGGGSGGGGS

SEQ ID NO: 8 - protein, 6 aa, Artificial Sequence
  4N
GSNNNN

SEQ ID NO: 9 - protein, 10 aa, Artificial Sequence
  8N
GSNNNNNNNN

SEQ ID NO: 10 - protein, 10 aa, Artificial Sequence
  LE8N
LENNNNNNNN

SEQ ID NO: 11 - protein, 31 aa, Artificial Sequence
  PRIMER
AATAAAACATATGGTAGACAACAAATTCAAC

SEQ ID NO: 12 - protein, 33 aa, Artificial Sequence
  PRIMER
ATTCTCGAGTTAATCATCATCATCATCATCTTC

SEQ ID NO: 13 - protein, 58 aa, Artificial Sequence [sequence omitted]

SEQ ID NO: 14 - protein, 290 aa, Artificial Sequence
  (Z)5
VDNKFNKEQQNAFYEILHLPNLNEEQRNAFIQSLKDDPSQSANLLAEAKKLNDAQAPKVDNKFNKEQQNAFYEILHLPNLNEEQRNAFIQSLKDDPSQSANLLAEAKKLNDAQAPKVDNKFNKEQQNAFYEILHLPNLNEEQRNAFIQSLKDDPSQSANLLAEAKKLNDAQAPKVDNKFNKEQQNAFYEILHLPNLNEEQRNAFIQSLKDDPSQSANLLAEAKKLNDAQAPKVDNKFNKEQQNAFYEILHLPNLNEEQRNAFIQSLKDDPSQSANLLAEAKKLNDAQAPK